European Patent Specification EP 3 608 337 B1, published April 17, 2024. Title: Bispecific T cell activating antigen binding molecules. Applicant: F. Hoffmann-La Roche AG. The sequence listing filed with the application follows.

SEQUENCE LISTING (68 sequences)

SEQ ID NO: 1 - protein, 207 aa, Homo sapiens
MQSGTHWRVLGLCLLSVGVWGQDGNEEMGGITQTPYKVSISGTTVILTCPQYPGSEILWQHNDKNIGGDEDDKNIGSDEDHLSLKEFSELEQSGYYVCYPRGSKPEDANFYLYLRARVCENCMEMDVMSVATIVIVDICITGGLLLLVYYWSKNRKAKAKPVTRGAGAGGRQRGQNKERPPPVPNPDYEPIRKGQRDLYSGLNQRRI

SEQ ID NO: 2 - protein, 198 aa, Macaca fascicularis
MQSGTRWRVLGLCLLSIGVWGQDGNEEMGSITQTPYQVSISGTTVILTCSQHLGSEAQWQHNGKNKEDSGDRLFLPEFSEMEQSGYYVCYPRGSNPEDASHHLYLKARVCENCMEMDVMAVATIVIVDICITLGLLLLVYYWSKNRKAKAKPVTRGAGAGGRQRGQNKERPPPVPNPDYEPIRKGQQDLYSGLNQRRI

SEQ ID NO: 3 - protein, 125 aa, Artificial Sequence
  CD3 VH
EVQLLESGGGLVQPGGSLRLSCAASGFTFSTYAMNWVRQAPGKGLEWVSRIRSKYNNYATYYADSVKGRFTISRDDSKNTLYLQMNSLRAEDTAVYYCVRHGNFGNSYVSWFAYWGQGTLVTVSS

SEQ ID NO: 4 - protein, 5 aa, Artificial Sequence
  CD3 HCDR1
TYAMN

SEQ ID NO: 5 - protein, 19 aa, Artificial Sequence
  CD3 HCDR2
RIRSKYNNYATYYADSVKG

SEQ ID NO: 6 - protein, 14 aa, Artificial Sequence
  CD3 HCDR3
HGNFGNSYVSWFAY

SEQ ID NO: 7 - protein, 109 aa, Artificial Sequence
  CD3 VL
QAVVTQEPSLTVSPGGTVTLTCGSSTGAVTTSNYANWVQEKPGQAFRGLIGGTNKRAPGTPARFSGSLLGGKAALTLSGAQPEDEAEYYCALWYSNLWVFGGGTKLTVL

SEQ ID NO: 8 - protein, 14 aa, Artificial Sequence
  CD3 LCDR1
GSSTGAVTTSNYAN

SEQ ID NO: 9 - protein, 7 aa, Artificial Sequence
  CD3 LCDR2
GTNKRAP

SEQ ID NO: 10 - protein, 9 aa, Artificial Sequence
  CD3 LCDR3
ALWYSNLWV

SEQ ID NO: 11 - protein, 10 aa, Artificial Sequence
  linker
GGGGSGGGGS

SEQ ID NO: 12 - protein, 11 aa, Artificial Sequence
  linker
DGGGGSGGGGS

SEQ ID NO: 13 - protein, 225 aa, Homo sapiens
DKTHTCPPCPAPELLGGPSVFLFPPKPKDTLMISRTPEVTCVVVDVSHEDPEVKFNWYVDGVEVHNAKTKPREEQYNSTYRVVSVLTVLHQDWLNGKEYKCKVSNKALPAPIEKTISKAKGQPREPQVYTLPPSRDELTKNQVSLTCLVKGFYPSDIAVEWESNGQPENNYKTTPPVLDSDGSFFLYSKLTVDKSRWQQGNVFSCSVMHEALHNHYTQKSLSLSP

SEQ ID NO: 14 - protein, 690 aa, Artificial Sequence
  CD20 VH-CH1-CD3 VH-CL-Fc (knob, P329G LALA)
QVQLVQSGAEVKKPGSSVKVSCKASGYAFSYSWINWVRQAPGQGLEWMGRIFPGDGDTDYNGKFKGRVTITADKSTSTAYMELSSLRSEDTAVYYCARNVFDGYWLVYWGQGTLVTVSSASTKGPSVFPLAPSSKSTSGGTAALGCLVKDYFPEPVTVSWNSGALTSGVHTFPAVLQSSGLYSLSSVVTVPSSSLGTQTYICNVNHKPSNTKVDKKVEPKSCDGGGGSGGGGSEVQLLESGGGLVQPGGSLRLSCAASGFTFSTYAMNWVRQAPGKGLEWVSRIRSKYNNYATYYADSVKGRFTISRDDSKNTLYLQMNSLRAEDTAVYYCVRHGNFGNSYVSWFAYWGQGTLVTVSSASVAAPSVFIFPPSDEQLKSGTASVVCLLNNFYPREAKVQWKVDNALQSGNSQESVTEQDSKDSTYSLSSTLTLSKADYEKHKVYACEVTHQGLSSPVTKSFNRGECDKTHTCPPCPAPEAAGGPSVFLFPPKPKDTLMISRTPEVTCVVVDVSHEDPEVKFNWYVDGVEVHNAKTKPREEQYNSTYRVVSVLTVLHQDWLNGKEYKCKVSNKALGAPIEKTISKAKGQPREPQVYTLPPCRDELTKNQVSLWCLVKGFYPSDIAVEWESNGQPENNYKTTPPVLDSDGSFFLYSKLTVDKSRWQQGNVFSCSVMHEALHNHYTQKSLSLSP

SEQ ID NO: 15 - protein, 447 aa, Artificial Sequence
  CD20 VH-CH1-Fc (hole, P329G LALA)
QVQLVQSGAEVKKPGSSVKVSCKASGYAFSYSWINWVRQAPGQGLEWMGRIFPGDGDTDYNGKFKGRVTITADKSTSTAYMELSSLRSEDTAVYYCARNVFDGYWLVYWGQGTLVTVSSASTKGPSVFPLAPSSKSTSGGTAALGCLVKDYFPEPVTVSWNSGALTSGVHTFPAVLQSSGLYSLSSVVTVPSSSLGTQTYICNVNHKPSNTKVDKKVEPKSCDKTHTCPPCPAPEAAGGPSVFLFPPKPKDTLMISRTPEVTCVVVDVSHEDPEVKFNWYVDGVEVHNAKTKPREEQYNSTYRVVSVLTVLHQDWLNGKEYKCKVSNKALGAPIEKTISKAKGQPREPQVCTLPPSRDELTKNQVSLSCAVKGFYPSDIAVEWESNGQPENNYKTTPPVLDSDGSFFLVSKLTVDKSRWQQGNVFSCSVMHEALHNHYTQKSLSLSP

SEQ ID NO: 16 - protein, 214 aa, Artificial Sequence
  CD3 VL-CH1
QAVVTQEPSLTVSPGGTVTLTCGSSTGAVTTSNYANWVQEKPGQAFRGLIGGTNKRAPGTPARFSGSLLGGKAALTLSGAQPEDEAEYYCALWYSNLWVFGGGTKLTVLSSASTKGPSVFPLAPSSKSTSGGTAALGCLVKDYFPEPVTVSWNSGALTSGVHTFPAVLQSSGLYSLSSVVTVPSSSLGTQTYICNVNHKPSNTKVDKKVEPKSC

SEQ ID NO: 17 - protein, 219 aa, Artificial Sequence
  CD20 VL-CL
DIVMTQTPLSLPVTPGEPASISCRSSKSLLHSNGITYLYWYLQKPGQSPQLLIYQMSNLVSGVPDRFSGSGSGTDFTLKISRVEAEDVGVYYCAQNLELPYTFGGGTKVEIKRTVAAPSVFIFPPSDEQLKSGTASVVCLLNNFYPREAKVQWKVDNALQSGNSQESVTEQDSKDSTYSLSSTLTLSKADYEKHKVYACEVTHQGLSSPVTKSFNRGEC

SEQ ID NO: 18 - protein, 672 aa, Artificial Sequence
  CD20 VH-CH1(EE)-CD3 VL-CH1-Fc (knob, P329G LALA)
QVQLVQSGAEVKKPGSSVKVSCKASGYAFSYSWINWVRQAPGQGLEWMGRIFPGDGDTDYNGKFKGRVTITADKSTSTAYMELSSLRSEDTAVYYCARNVFDGYWLVYWGQGTLVTVSSASTKGPSVFPLAPSSKSTSGGTAALGCLVEDYFPEPVTVSWNSGALTSGVHTFPAVLQSSGLYSLSSVVTVPSSSLGTQTYICNVNHKPSNTKVDEKVEPKSCDGGGGSGGGGSQAVVTQEPSLTVSPGGTVTLTCGSSTGAVTTSNYANWVQEKPGQAFRGLIGGTNKRAPGTPARFSGSLLGGKAALTLSGAQPEDEAEYYCALWYSNLWVFGGGTKLTVLSSASTKGPSVFPLAPSSKSTSGGTAALGCLVKDYFPEPVTVSWNSGALTSGVHTFPAVLQSSGLYSLSSVVTVPSSSLGTQTYICNVNHKPSNTKVDKKVEPKSCDKTHTCPPCPAPEAAGGPSVFLFPPKPKDTLMISRTPEVTCVVVDVSHEDPEVKFNWYVDGVEVHNAKTKPREEQYNSTYRVVSVLTVLHQDWLNGKEYKCKVSNKALGAPIEKTISKAKGQPREPQVYTLPPCRDELTKNQVSLWCLVKGFYPSDIAVEWESNGQPENNYKTTPPVLDSDGSFFLYSKLTVDKSRWQQGNVFSCSVMHEALHNHYTQKSLSLSP

SEQ ID NO: 19 - protein, 447 aa, Artificial Sequence
  CD20 VH-CH1(EE)-Fc (hole, P329G LALA)
QVQLVQSGAEVKKPGSSVKVSCKASGYAFSYSWINWVRQAPGQGLEWMGRIFPGDGDTDYNGKFKGRVTITADKSTSTAYMELSSLRSEDTAVYYCARNVFDGYWLVYWGQGTLVTVSSASTKGPSVFPLAPSSKSTSGGTAALGCLVEDYFPEPVTVSWNSGALTSGVHTFPAVLQSSGLYSLSSVVTVPSSSLGTQTYICNVNHKPSNTKVDEKVEPKSCDKTHTCPPCPAPEAAGGPSVFLFPPKPKDTLMISRTPEVTCVVVDVSHEDPEVKFNWYVDGVEVHNAKTKPREEQYNSTYRVVSVLTVLHQDWLNGKEYKCKVSNKALGAPIEKTISKAKGQPREPQVCTLPPSRDELTKNQVSLSCAVKGFYPSDIAVEWESNGQPENNYKTTPPVLDSDGSFFLVSKLTVDKSRWQQGNVFSCSVMHEALHNHYTQKSLSLSP

SEQ ID NO: 20 - protein, 219 aa, Artificial Sequence
  CD20 VL-CL(RK)
DIVMTQTPLSLPVTPGEPASISCRSSKSLLHSNGITYLYWYLQKPGQSPQLLIYQMSNLVSGVPDRFSGSGSGTDFTLKISRVEAEDVGVYYCAQNLELPYTFGGGTKVEIKRTVAAPSVFIFPPSDRKLKSGTASVVCLLNNFYPREAKVQWKVDNALQSGNSQESVTEQDSKDSTYSLSSTLTLSKADYEKHKVYACEVTHQGLSSPVTKSFNRGEC

SEQ ID NO: 21 - protein, 232 aa, Artificial Sequence
  CD3 VH-CL
EVQLLESGGGLVQPGGSLRLSCAASGFTFSTYAMNWVRQAPGKGLEWVSRIRSKYNNYATYYADSVKGRFTISRDDSKNTLYLQMNSLRAEDTAVYYCVRHGNFGNSYVSWFAYWGQGTLVTVSSASVAAPSVFIFPPSDEQLKSGTASVVCLLNNFYPREAKVQWKVDNALQSGNSQESVTEQDSKDSTYSLSSTLTLSKADYEKHKVYACEVTHQGLSSPVTKSFNRGEC

SEQ ID NO: 22 - protein, 687 aa, Artificial Sequence
  BCMA VH-CH1-CD3 VH-CL-Fc (knob, P329G LALA)
EVQLLESGGGLVQPGGSLRLSCAASGFTFSSYAMSWVRQAPGKGLEWVSAISGSGGSTYYADSVKGRFTISRDNSKNTLYLQMNSLRAEDTAVYYCAKVLGWFDYWGQGTLVTVSSASTKGPSVFPLAPSSKSTSGGTAALGCLVKDYFPEPVTVSWNSGALTSGVHTFPAVLQSSGLYSLSSVVTVPSSSLGTQTYICNVNHKPSNTKVDKKVEPKSCDGGGGSGGGGSEVQLLESGGGLVQPGGSLRLSCAASGFTFSTYAMNWVRQAPGKGLEWVSRIRSKYNNYATYYADSVKGRFTISRDDSKNTLYLQMNSLRAEDTAVYYCVRHGNFGNSYVSWFAYWGQGTLVTVSSASVAAPSVFIFPPSDEQLKSGTASVVCLLNNFYPREAKVQWKVDNALQSGNSQESVTEQDSKDSTYSLSSTLTLSKADYEKHKVYACEVTHQGLSSPVTKSFNRGECDKTHTCPPCPAPEAAGGPSVFLFPPKPKDTLMISRTPEVTCVVVDVSHEDPEVKFNWYVDGVEVHNAKTKPREEQYNSTYRVVSVLTVLHQDWLNGKEYKCKVSNKALGAPIEKTISKAKGQPREPQVYTLPPCRDELTKNQVSLWCLVKGFYPSDIAVEWESNGQPENNYKTTPPVLDSDGSFFLYSKLTVDKSRWQQGNVFSCSVMHEALHNHYTQKSLSLSP

SEQ ID NO: 23 - protein, 444 aa, Artificial Sequence
  BCMA VH-CH1-Fc (hole, P329G LALA)
EVQLLESGGGLVQPGGSLRLSCAASGFTFSSYAMSWVRQAPGKGLEWVSAISGSGGSTYYADSVKGRFTISRDNSKNTLYLQMNSLRAEDTAVYYCAKVLGWFDYWGQGTLVTVSSASTKGPSVFPLAPSSKSTSGGTAALGCLVKDYFPEPVTVSWNSGALTSGVHTFPAVLQSSGLYSLSSVVTVPSSSLGTQTYICNVNHKPSNTKVDKKVEPKSCDKTHTCPPCPAPEAAGGPSVFLFPPKPKDTLMISRTPEVTCVVVDVSHEDPEVKFNWYVDGVEVHNAKTKPREEQYNSTYRVVSVLTVLHQDWLNGKEYKCKVSNKALGAPIEKTISKAKGQPREPQVCTLPPSRDELTKNQVSLSCAVKGFYPSDIAVEWESNGQPENNYKTTPPVLDSDGSFFLVSKLTVDKSRWQQGNVFSCSVMHEALHNHYTQKSLSLSP

SEQ ID NO: 24 - protein, 214 aa, Artificial Sequence; identical to SEQ ID NO: 16
  CD3 VL-CH1

SEQ ID NO: 25 - protein, 216 aa, Artificial Sequence
  BCMA VL-CL
EIVLTQSPGTLSLSPGERATLSCRASQSVSSSYLAWYQQKPGQAPRLLIYGASSRATGIPDRFSGSGSGTDFTLTISRLEPEDFAVYYCQQYGYPPDFTFGQGTKVEIKRTVAAPSVFIFPPSDEQLKSGTASVVCLLNNFYPREAKVQWKVDNALQSGNSQESVTEQDSKDSTYSLSSTLTLSKADYEKHKVYACEVTHQGLSSPVTKSFNRGEC

SEQ ID NO: 26 - protein, 669 aa, Artificial Sequence
  BCMA VH-CH1(EE)-CD3 VL-CH1-Fc (knob, P329G LALA)
EVQLLESGGGLVQPGGSLRLSCAASGFTFSSYAMSWVRQAPGKGLEWVSAISGSGGSTYYADSVKGRFTISRDNSKNTLYLQMNSLRAEDTAVYYCAKVLGWFDYWGQGTLVTVSSASTKGPSVFPLAPSSKSTSGGTAALGCLVEDYFPEPVTVSWNSGALTSGVHTFPAVLQSSGLYSLSSVVTVPSSSLGTQTYICNVNHKPSNTKVDEKVEPKSCDGGGGSGGGGSQAVVTQEPSLTVSPGGTVTLTCGSSTGAVTTSNYANWVQEKPGQAFRGLIGGTNKRAPGTPARFSGSLLGGKAALTLSGAQPEDEAEYYCALWYSNLWVFGGGTKLTVLSSASTKGPSVFPLAPSSKSTSGGTAALGCLVKDYFPEPVTVSWNSGALTSGVHTFPAVLQSSGLYSLSSVVTVPSSSLGTQTYICNVNHKPSNTKVDKKVEPKSCDKTHTCPPCPAPEAAGGPSVFLFPPKPKDTLMISRTPEVTCVVVDVSHEDPEVKFNWYVDGVEVHNAKTKPREEQYNSTYRVVSVLTVLHQDWLNGKEYKCKVSNKALGAPIEKTISKAKGQPREPQVYTLPPCRDELTKNQVSLWCLVKGFYPSDIAVEWESNGQPENNYKTTPPVLDSDGSFFLYSKLTVDKSRWQQGNVFSCSVMHEALHNHYTQKSLSLSP

SEQ ID NO: 27 - protein, 444 aa, Artificial Sequence
  BCMA VH-CH1(EE)-Fc (hole, P329G LALA)
EVQLLESGGGLVQPGGSLRLSCAASGFTFSSYAMSWVRQAPGKGLEWVSAISGSGGSTYYADSVKGRFTISRDNSKNTLYLQMNSLRAEDTAVYYCAKVLGWFDYWGQGTLVTVSSASTKGPSVFPLAPSSKSTSGGTAALGCLVEDYFPEPVTVSWNSGALTSGVHTFPAVLQSSGLYSLSSVVTVPSSSLGTQTYICNVNHKPSNTKVDEKVEPKSCDKTHTCPPCPAPEAAGGPSVFLFPPKPKDTLMISRTPEVTCVVVDVSHEDPEVKFNWYVDGVEVHNAKTKPREEQYNSTYRVVSVLTVLHQDWLNGKEYKCKVSNKALGAPIEKTISKAKGQPREPQVCTLPPSRDELTKNQVSLSCAVKGFYPSDIAVEWESNGQPENNYKTTPPVLDSDGSFFLVSKLTVDKSRWQQGNVFSCSVMHEALHNHYTQKSLSLSP

SEQ ID NO: 28 - protein, 232 aa, Artificial Sequence; identical to SEQ ID NO: 21
  CD3 VH-CL

SEQ ID NO: 29 - protein, 216 aa, Artificial Sequence
  BCMA VL-CL(RK)
EIVLTQSPGTLSLSPGERATLSCRASQSVSSSYLAWYQQKPGQAPRLLIYGASSRATGIPDRFSGSGSGTDFTLTISRLEPEDFAVYYCQQYGYPPDFTFGQGTKVEIKRTVAAPSVFIFPPSDRKLKSGTASVVCLLNNFYPREAKVQWKVDNALQSGNSQESVTEQDSKDSTYSLSSTLTLSKADYEKHKVYACEVTHQGLSSPVTKSFNRGEC

SEQ ID NO: 30 - protein, 119 aa, Artificial Sequence
  CD20 VH
QVQLVQSGAEVKKPGSSVKVSCKASGYAFSYSWINWVRQAPGQGLEWMGRIFPGDGDTDYNGKFKGRVTITADKSTSTAYMELSSLRSEDTAVYYCARNVFDGYWLVYWGQGTLVTVSS

SEQ ID NO: 31 - protein, 115 aa, Artificial Sequence
  CD20 VL
DIVMTQTPLSLPVTPGEPASISCRSSKSLLHSNGITYLYWYLQKPGQSPQLLIYQMSNLVSGVPDRFSGSGSGTDFTLKISRVEAEDVGVYYCAQNLELPYTFGGGTKVEIKRTV

SEQ ID NO: 32 - protein, 672 aa, Artificial Sequence
  CD3 VL-CH1-CD20 VH-CH1(EE)-Fc(knob, P329G LALA)
QAVVTQEPSLTVSPGGTVTLTCGSSTGAVTTSNYANWVQEKPGQAFRGLIGGTNKRAPGTPARFSGSLLGGKAALTLSGAQPEDEAEYYCALWYSNLWVFGGGTKLTVLSSASTKGPSVFPLAPSSKSTSGGTAALGCLVKDYFPEPVTVSWNSGALTSGVHTFPAVLQSSGLYSLSSVVTVPSSSLGTQTYICNVNHKPSNTKVDKKVEPKSCDGGGGSGGGGSQVQLVQSGAEVKKPGSSVKVSCKASGYAFSYSWINWVRQAPGQGLEWMGRIFPGDGDTDYNGKFKGRVTITADKSTSTAYMELSSLRSEDTAVYYCARNVFDGYWLVYWGQGTLVTVSSASTKGPSVFPLAPSSKSTSGGTAALGCLVEDYFPEPVTVSWNSGALTSGVHTFPAVLQSSGLYSLSSVVTVPSSSLGTQTYICNVNHKPSNTKVDEKVEPKSCDKTHTCPPCPAPEAAGGPSVFLFPPKPKDTLMISRTPEVTCVVVDVSHEDPEVKFNWYVDGVEVHNAKTKPREEQYNSTYRVVSVLTVLHQDWLNGKEYKCKVSNKALGAPIEKTISKAKGQPREPQVYTLPPCRDELTKNQVSLWCLVKGFYPSDIAVEWESNGQPENNYKTTPPVLDSDGSFFLYSKLTVDKSRWQQGNVFSCSVMHEALHNHYTQKSLSLSP

SEQ ID NO: 33 - protein, 672 aa, Artificial Sequence
  CD20 VH-CH1-CD3 VL-CH1-Fc(knob, P329G LALA)
QVQLVQSGAEVKKPGSSVKVSCKASGYAFSYSWINWVRQAPGQGLEWMGRIFPGDGDTDYNGKFKGRVTITADKSTSTAYMELSSLRSEDTAVYYCARNVFDGYWLVYWGQGTLVTVSSASTKGPSVFPLAPSSKSTSGGTAALGCLVKDYFPEPVTVSWNSGALTSGVHTFPAVLQSSGLYSLSSVVTVPSSSLGTQTYICNVNHKPSNTKVDKKVEPKSCDGGGGSGGGGSQAVVTQEPSLTVSPGGTVTLTCGSSTGAVTTSNYANWVQEKPGQAFRGLIGGTNKRAPGTPARFSGSLLGGKAALTLSGAQPEDEAEYYCALWYSNLWVFGGGTKLTVLSSASTKGPSVFPLAPSSKSTSGGTAALGCLVKDYFPEPVTVSWNSGALTSGVHTFPAVLQSSGLYSLSSVVTVPSSSLGTQTYICNVNHKPSNTKVDKKVEPKSCDKTHTCPPCPAPEAAGGPSVFLFPPKPKDTLMISRTPEVTCVVVDVSHEDPEVKFNWYVDGVEVHNAKTKPREEQYNSTYRVVSVLTVLHQDWLNGKEYKCKVSNKALGAPIEKTISKAKGQPREPQVYTLPPCRDELTKNQVSLWCLVKGFYPSDIAVEWESNGQPENNYKTTPPVLDSDGSFFLYSKLTVDKSRWQQGNVFSCSVMHEALHNHYTQKSLSLSP

SEQ ID NO: 34 - protein, 676 aa, Artificial Sequence
  CD20 VH-CH1 CD3 VL-CL-Fc(knob, P329G LALA)
QVQLVQSGAEVKKPGSSVKVSCKASGYAFSYSWINWVRQAPGQGLEWMGRIFPGDGDTDYNGKFKGRVTITADKSTSTAYMELSSLRSEDTAVYYCARNVFDGYWLVYWGQGTLVTVSSASTKGPSVFPLAPSSKSTSGGTAALGCLVKDYFPEPVTVSWNSGALTSGVHTFPAVLQSSGLYSLSSVVTVPSSSLGTQTYICNVNHKPSNTKVDKKVEPKSCDGGGGSGGGGSQAVVTQEPSLTVSPGGTVTLTCGSSTGAVTTSNYANWVQEKPGQAFRGLIGGTNKRAPGTPARFSGSLLGGKAALTLSGAQPEDEAEYYCALWYSNLWVFGGGTKLTVLSSASVAAPSVFIFPPSDEQLKSGTASVVCLLNNFYPREAKVQWKVDNALQSGNSQESVTEQDSKDSTYSLSSTLTLSKADYEKHKVYACEVTHQGLSSPVTKSFNRGECDKTHTCPPCPAPEAAGGPSVFLFPPKPKDTLMISRTPEVTCVVVDVSHEDPEVKFNWYVDGVEVHNAKTKPREEQYNSTYRVVSVLTVLHQDWLNGKEYKCKVSNKALGAPIEKTISKAKGQPREPQVYTLPPCRDELTKNQVSLWCLVKGFYPSDIAVEWESNGQPENNYKTTPPVLDSDGSFFLYSKLTVDKSRWQQGNVFSCSVMHEALHNHYTQKSLSLSP

SEQ ID NO: 35 - protein, 228 aa, Artificial Sequence
  CD3 VH-CH1
EVQLLESGGGLVQPGGSLRLSCAASGFTFSTYAMNWVRQAPGKGLEWVSRIRSKYNNYATYYADSVKGRFTISRDDSKNTLYLQMNSLRAEDTAVYYCVRHGNFGNSYVSWFAYWGQGTLVTVSSASTKGPSVFPLAPSSKSTSGGTAALGCLVKDYFPEPVTVSWNSGALTSGVHTFPAVLQSSGLYSLSSVVTVPSSSLGTQTYICNVNHKPSNTKVDKKVEPKSC

SEQ ID NO: 36 - protein, 681 aa, Artificial Sequence
  CD20 VL-CH1-CD3 VH-CH1(EE)-Fc(knob, P329G LALA)
DIVMTQTPLSLPVTPGEPASISCRSSKSLLHSNGITYLYWYLQKPGQSPQLLIYQMSNLVSGVPDRFSGSGSGTDFTLKISRVEAEDVGVYYCAQNLELPYTFGGGTKVEIKSSASTKGPSVFPLAPSSKSTSGGTAALGCLVKDYFPEPVTVSWNSGALTSGVHTFPAVLQSSGLYSLSSVVTVPSSSLGTQTYICNVNHKPSNTKVDKKVEPKSCDGGGGSGGGGSEVQLLESGGGLVQPGGSLRLSCAASGFTFSTYAMNWVRQAPGKGLEWVSRIRSKYNNYATYYADSVKGRFTISRDDSKNTLYLQMNSLRAEDTAVYYCVRHGNFGNSYVSWFAYWGQGTLVTVSSASTKGPSVFPLAPSSKSTSGGTAALGCLVEDYFPEPVTVSWNSGALTSGVHTFPAVLQSSGLYSLSSVVTVPSSSLGTQTYICNVNHKPSNTKVDEKVEPKSCDKTHTCPPCPAPEAAGGPSVFLFPPKPKDTLMISRTPEVTCVVVDVSHEDPEVKFNWYVDGVEVHNAKTKPREEQYNSTYRVVSVLTVLHQDWLNGKEYKCKVSNKALGAPIEKTISKAKGQPREPQVYTLPPCRDELTKNQVSLWCLVKGFYPSDIAVEWESNGQPENNYKTTPPVLDSDGSFFLYSKLTVDKSRWQQGNVFSCSVMHEALHNHYTQKSLSLSP

SEQ ID NO: 37 - protein, 442 aa, Artificial Sequence
  CD20 VL-CH1-Fc(hole, P329G LALA)
DIVMTQTPLSLPVTPGEPASISCRSSKSLLHSNGITYLYWYLQKPGQSPQLLIYQMSNLVSGVPDRFSGSGSGTDFTLKISRVEAEDVGVYYCAQNLELPYTFGGGTKVEIKSSASTKGPSVFPLAPSSKSTSGGTAALGCLVKDYFPEPVTVSWNSGALTSGVHTFPAVLQSSGLYSLSSVVTVPSSSLGTQTYICNVNHKPSNTKVDKKVEPKSCDKTHTCPPCPAPEAAGGPSVFLFPPKPKDTLMISRTPEVTCVVVDVSHEDPEVKFNWYVDGVEVHNAKTKPREEQYNSTYRVVSVLTVLHQDWLNGKEYKCKVSNKALGAPIEKTISKAKGQPREPQVCTLPPSRDELTKNQVSLSCAVKGFYPSDIAVEWESNGQPENNYKTTPPVLDSDGSFFLVSKLTVDKSRWQQGNVFSCSVMHEALHNHYTQKSLSLSP

SEQ ID NO: 38 - protein, 215 aa, Artificial Sequence
  CD3 VL-CL(KK)
QAVVTQEPSLTVSPGGTVTLTCGSSTGAVTTSNYANWVQEKPGQAFRGLIGGTNKRAPGTPARFSGSLLGGKAALTLSGAQPEDEAEYYCALWYSNLWVFGGGTKLTVLGQPKAAPSVTLFPPSSKKLQANKATLVCLISDFYPGAVTVAWKADSSPVKAGVETTTPSKQSNNKYAASSYLSLTPEQWKSHRSYSCQVTHEGSTVEKTVAPTECS

SEQ ID NO: 39 - protein, 226 aa, Artificial Sequence
  CD20 VH-CL
QVQLVQSGAEVKKPGSSVKVSCKASGYAFSYSWINWVRQAPGQGLEWMGRIFPGDGDTDYNGKFKGRVTITADKSTSTAYMELSSLRSEDTAVYYCARNVFDGYWLVYWGQGTLVTVSSASVAAPSVFIFPPSDEQLKSGTASVVCLLNNFYPREAKVQWKVDNALQSGNSQESVTEQDSKDSTYSLSSTLTLSKADYEKHKVYACEVTHQGLSSPVTKSFNRGEC

SEQ ID NO: 40 - protein, 672 aa, Artificial Sequence
  CD20 VH-CH1(EE)-CD3 VL-CH1-Fc(DD, P329G LALA)
QVQLVQSGAEVKKPGSSVKVSCKASGYAFSYSWINWVRQAPGQGLEWMGRIFPGDGDTDYNGKFKGRVTITADKSTSTAYMELSSLRSEDTAVYYCARNVFDGYWLVYWGQGTLVTVSSASTKGPSVFPLAPSSKSTSGGTAALGCLVEDYFPEPVTVSWNSGALTSGVHTFPAVLQSSGLYSLSSVVTVPSSSLGTQTYICNVNHKPSNTKVDEKVEPKSCDGGGGSGGGGSQAVVTQEPSLTVSPGGTVTLTCGSSTGAVTTSNYANWVQEKPGQAFRGLIGGTNKRAPGTPARFSGSLLGGKAALTLSGAQPEDEAEYYCALWYSNLWVFGGGTKLTVLSSASTKGPSVFPLAPSSKSTSGGTAALGCLVKDYFPEPVTVSWNSGALTSGVHTFPAVLQSSGLYSLSSVVTVPSSSLGTQTYICNVNHKPSNTKVDKKVEPKSCDKTHTCPPCPAPEAAGGPSVFLFPPKPKDTLMISRTPEVTCVVVDVSHEDPEVKFNWYVDGVEVHNAKTKPREEQYNSTYRVVSVLTVLHQDWLNGKEYKCKVSNKALGAPIEKTISKAKGQPREPQVYTLPPSRDELTKNQVSLTCLVKGFYPSDIAVEWESNGQPENNYDTTPPVLDSDGSFFLYSDLTVDKSRWQQGNVFSCSVMHEALHNHYTQKSLSLSP

SEQ ID NO: 41 - protein, 447 aa, Artificial Sequence
  CD20 VH-CH1(EE)-Fc(KK, P329G LALA)
QVQLVQSGAEVKKPGSSVKVSCKASGYAFSYSWINWVRQAPGQGLEWMGRIFPGDGDTDYNGKFKGRVTITADKSTSTAYMELSSLRSEDTAVYYCARNVFDGYWLVYWGQGTLVTVSSASTKGPSVFPLAPSSKSTSGGTAALGCLVEDYFPEPVTVSWNSGALTSGVHTFPAVLQSSGLYSLSSVVTVPSSSLGTQTYICNVNHKPSNTKVDEKVEPKSCDKTHTCPPCPAPEAAGGPSVFLFPPKPKDTLMISRTPEVTCVVVDVSHEDPEVKFNWYVDGVEVHNAKTKPREEQYNSTYRVVSVLTVLHQDWLNGKEYKCKVSNKALGAPIEKTISKAKGQPREPQVYTLPPSRKELTKNQVSLTCLVKGFYPSDIAVEWESNGQPENNYKTTPPVLKSDGSFFLYSKLTVDKSRWQQGNVFSCSVMHEALHNHYTQKSLSLSP

SEQ ID NO: 42 - protein, 447 aa, Artificial Sequence
  CD20 VH-CH1(EE)-Fc(hole, N297G)
QVQLVQSGAEVKKPGSSVKVSCKASGYAFSYSWINWVRQAPGQGLEWMGRIFPGDGDTDYNGKFKGRVTITADKSTSTAYMELSSLRSEDTAVYYCARNVFDGYWLVYWGQGTLVTVSSASTKGPSVFPLAPSSKSTSGGTAALGCLVEDYFPEPVTVSWNSGALTSGVHTFPAVLQSSGLYSLSSVVTVPSSSLGTQTYICNVNHKPSNTKVDEKVEPKSCDKTHTCPPCPAPELLGGPSVFLFPPKPKDTLMISRTPEVTCVVVDVSHEDPEVKFNWYVDGVEVHNAKTKPREEQYGSTYRVVSVLTVLHQDWLNGKEYKCKVSNKALPAPIEKTISKAKGQPREPQVCTLPPSRDELTKNQVSLSCAVKGFYPSDIAVEWESNGQPENNYKTTPPVLDSDGSFFLVSKLTVDKSRWQQGNVFSCSVMHEALHNHYTQKSLSLSP

SEQ ID NO: 43 - protein, 439 aa, Artificial Sequence
  CD3 VL-CH1-Fc(knob, N297G)
QAVVTQEPSLTVSPGGTVTLTCGSSTGAVTTSNYANWVQEKPGQAFRGLIGGTNKRAPGTPARFSGSLLGGKAALTLSGAQPEDEAEYYCALWYSNLWVFGGGTKLTVLSSASTKGPSVFPLAPSSKSTSGGTAALGCLVKDYFPEPVTVSWNSGALTSGVHTFPAVLQSSGLYSLSSVVTVPSSSLGTQTYICNVNHKPSNTKVDKKVEPKSCDKTHTCPPCPAPELLGGPSVFLFPPKPKDTLMISRTPEVTCVVVDVSHEDPEVKFNWYVDGVEVHNAKTKPREEQYGSTYRVVSVLTVLHQDWLNGKEYKCKVSNKALPAPIEKTISKAKGQPREPQVYTLPPCRDELTKNQVSLWCLVKGFYPSDIAVEWESNGQPENNYKTTPPVLDSDGSFFLYSKLTVDKSRWQQGNVFSCSVMHEALHNHYTQKSLSLSP

SEQ ID NO: 44 - protein, 450 aa, Artificial Sequence
  CD20 VH-CH1(EE)-Fc(hole, N297G)
EVQLVESGGGLVQPGGSLRLSCAASGYTFTSYNMHWVRQAPGKGLEWVGAIYPGNGDTSYNQKFKGRFTISVDKSKNTLYLQMNSLRAEDTAVYYCARVVYYSNSYWYFDVWGQGTLVTVSSASTKGPSVFPLAPSSKSTSGGTAALGCLVEDYFPEPVTVSWNSGALTSGVHTFPAVLQSSGLYSLSSVVTVPSSSLGTQTYICNVNHKPSNTKVDEKVEPKSCDKTHTCPPCPAPELLGGPSVFLFPPKPKDTLMISRTPEVTCVVVDVSHEDPEVKFNWYVDGVEVHNAKTKPREEQYGSTYRVVSVLTVLHQDWLNGKEYKCKVSNKALPAPIEKTISKAKGQPREPQVCTLPPSRDELTKNQVSLSCAVKGFYPSDIAVEWESNGQPENNYKTTPPVLDSDGSFFLVSKLTVDKSRWQQGNVFSCSVMHEALHNHYTQKSLSLSP

SEQ ID NO: 45 - protein, 213 aa, Artificial Sequence
  CD20 VL-CL(RK)
DIQMTQSPSSLSASVGDRVTITCRASSSVSYMHWYQQKPGKAPKPLIYAPSNLASGVPSRFSGSGSGTDFTLTISSLQPEDFATYYCQQWSFNPPTFGQGTKVEIKRTVAAPSVFIFPPSDRKLKSGTASVVCLLNNFYPREAKVQWKVDNALQSGNSQESVTEQDSKDSTYSLSSTLTLSKADYEKHKVYACEVTHQGLSSPVTKSFNRGEC

SEQ ID NO: 46 - protein, 5 aa, Artificial Sequence
  CD20 HCDR1
YSWIN

SEQ ID NO: 47 - protein, 17 aa, Artificial Sequence
  CD20 HCDR2
RIFPGDGDTDYNGKFKG

SEQ ID NO: 48 - protein, 10 aa, Artificial Sequence
  CD20 HCDR3
NVFDGYWLVY

SEQ ID NO: 49 - protein, 16 aa, Artificial Sequence
  CD20 LCDR1
RSSKSLLHSNGITYLY

SEQ ID NO: 50 - protein, 7 aa, Artificial Sequence
  CD20 LCDR2
QMSNLVS

SEQ ID NO: 51 - protein, 9 aa, Artificial Sequence
  CD20 LCDR3
AQNLELPYT

SEQ ID NO: 52 - protein, 673 aa, Artificial Sequence
  Her2 VH-CH1(EE)-CD3 VL-CH1-Fc(knob, P329G LALA)
EVQLVESGGGLVQPGGSLRLSCAASGFNIKDTYIHWVRQAPGKGLEWVARIYPTNGYTRYADSVKGRFTISADTSKNTAYLQMNSLRAEDTAVYYCSRWGGDGFYAMDYWGQGTLVTVSSASTKGPSVFPLAPSSKSTSGGTAALGCLVEDYFPEPVTVSWNSGALTSGVHTFPAVLQSSGLYSLSSVVTVPSSSLGTQTYICNVNHKPSNTKVDEKVEPKSCDGGGGSGGGGSQAVVTQEPSLTVSPGGTVTLTCGSSTGAVTTSNYANWVQEKPGQAFRGLIGGTNKRAPGTPARFSGSLLGGKAALTLSGAQPEDEAEYYCALWYSNLWVFGGGTKLTVLSSASTKGPSVFPLAPSSKSTSGGTAALGCLVKDYFPEPVTVSWNSGALTSGVHTFPAVLQSSGLYSLSSVVTVPSSSLGTQTYICNVNHKPSNTKVDKKVEPKSCDKTHTCPPCPAPEAAGGPSVFLFPPKPKDTLMISRTPEVTCVVVDVSHEDPEVKFNWYVDGVEVHNAKTKPREEQYNSTYRVVSVLTVLHQDWLNGKEYKCKVSNKALGAPIEKTISKAKGQPREPQVYTLPPCRDELTKNQVSLWCLVKGFYPSDIAVEWESNGQPENNYKTTPPVLDSDGSFFLYSKLTVDKSRWQQGNVFSCSVMHEALHNHYTQKSLSLSP

SEQ ID NO: 53 - protein, 448 aa, Artificial Sequence
  Her2 VH-CH1(EE)-Fc(hole, P329G LALA)
EVQLVESGGGLVQPGGSLRLSCAASGFNIKDTYIHWVRQAPGKGLEWVARIYPTNGYTRYADSVKGRFTISADTSKNTAYLQMNSLRAEDTAVYYCSRWGGDGFYAMDYWGQGTLVTVSSASTKGPSVFPLAPSSKSTSGGTAALGCLVEDYFPEPVTVSWNSGALTSGVHTFPAVLQSSGLYSLSSVVTVPSSSLGTQTYICNVNHKPSNTKVDEKVEPKSCDKTHTCPPCPAPEAAGGPSVFLFPPKPKDTLMISRTPEVTCVVVDVSHEDPEVKFNWYVDGVEVHNAKTKPREEQYNSTYRVVSVLTVLHQDWLNGKEYKCKVSNKALGAPIEKTISKAKGQPREPQVCTLPPSRDELTKNQVSLSCAVKGFYPSDIAVEWESNGQPENNYKTTPPVLDSDGSFFLVSKLTVDKSRWQQGNVFSCSVMHEALHNHYTQKSLSLSP

SEQ ID NO: 54 - protein, 214 aa, Artificial Sequence
  Her2 VL-CL(RK)
DIQMTQSPSSLSASVGDRVTITCRASQDVNTAVAWYQQKPGKAPKLLIYSASFLYSGVPSRFSGSRSGTDFTLTISSLQPEDFATYYCQQHYTTPPTFGQGTKVEIKRTVAAPSVFIFPPSDRKLKSGTASVVCLLNNFYPREAKVQWKVDNALQSGNSQESVTEQDSKDSTYSLSSTLTLSKADYEKHKVYACEVTHQGLSSPVTKSFNRGEC

SEQ ID NO: 55 - protein, 673 aa, Artificial Sequence
  CD3 VL-CH1-Her3 VH-CH1(EE)- Fc(knob, P329G LALA)
QAVVTQEPSLTVSPGGTVTLTCGSSTGAVTTSNYANWVQEKPGQAFRGLIGGTNKRAPGTPARFSGSLLGGKAALTLSGAQPEDEAEYYCALWYSNLWVFGGGTKLTVLSSASTKGPSVFPLAPSSKSTSGGTAALGCLVKDYFPEPVTVSWNSGALTSGVHTFPAVLQSSGLYSLSSVVTVPSSSLGTQTYICNVNHKPSNTKVDKKVEPKSCDGGGGSGGGGSQVQLVQSGAEVKKPGASVKVSCKASGYTFRSSYISWVRQAPGQGLEWMGWIYAGTGSPSYNQKLQGRVTMTTDTSTSTAYMELRSLRSDDTAVYYCARHRDYYSNSLTYWGQGTLVTVSSASTKGPSVFPLAPSSKSTSGGTAALGCLVEDYFPEPVTVSWNSGALTSGVHTFPAVLQSSGLYSLSSVVTVPSSSLGTQTYICNVNHKPSNTKVDEKVEPKSCDKTHTCPPCPAPEAAGGPSVFLFPPKPKDTLMISRTPEVTCVVVDVSHEDPEVKFNWYVDGVEVHNAKTKPREEQYNSTYRVVSVLTVLHQDWLNGKEYKCKVSNKALGAPIEKTISKAKGQPREPQVYTLPPCRDELTKNQVSLWCLVKGFYPSDIAVEWESNGQPENNYKTTPPVLDSDGSFFLYSKLTVDKSRWQQGNVFSCSVMHEALHNHYTQKSLSLSP

SEQ ID NO: 56 - protein, 448 aa, Artificial Sequence
  Her3 VH-CH1(EE)-Fc(hole, P329G LALA)
QVQLVQSGAEVKKPGASVKVSCKASGYTFRSSYISWVRQAPGQGLEWMGWIYAGTGSPSYNQKLQGRVTMTTDTSTSTAYMELRSLRSDDTAVYYCARHRDYYSNSLTYWGQGTLVTVSSASTKGPSVFPLAPSSKSTSGGTAALGCLVEDYFPEPVTVSWNSGALTSGVHTFPAVLQSSGLYSLSSVVTVPSSSLGTQTYICNVNHKPSNTKVDEKVEPKSCDKTHTCPPCPAPEAAGGPSVFLFPPKPKDTLMISRTPEVTCVVVDVSHEDPEVKFNWYVDGVEVHNAKTKPREEQYNSTYRVVSVLTVLHQDWLNGKEYKCKVSNKALGAPIEKTISKAKGQPREPQVCTLPPSRDELTKNQVSLSCAVKGFYPSDIAVEWESNGQPENNYKTTPPVLDSDGSFFLVSKLTVDKSRWQQGNVFSCSVMHEALHNHYTQKSLSLSP

SEQ ID NO: 57 - protein, 220 aa, Artificial Sequence
  Her3 VL-CL
DIVMTQSPDSLAVSLGERATINCKSSQSVLNSGNQKNYLTWYQQKPGQPPKLLIYWASTRESGVPDRFSGSGSGTDFTLTISSLQAEDVAVYYCQSDYSYPYTFGQGTKLEIKRTVAAPSVFIFPPSDRKLKSGTASVVCLLNNFYPREAKVQWKVDNALQSGNSQESVTEQDSKDSTYSLSSTLTLSKADYEKHKVYACEVTHQGLSSPVTKSFNRGEC

SEQ ID NO: 58 - protein, 664 aa, Artificial Sequence
  MCSP VH-CH1(EE)-MCSP VH-CH1(EE)-CD3 VL-CH1
EVQLQESGPGLVKPSQSLSLTCSVTGYSITSGYYWNWIRQFPGNKLEWMGYITYDGSNNYNPSLKNRISITRDTSKNQFFLKLNSVTTEDTATYYCADFDYWGQGTTLTVSSASTKGPSVFPLAPSSKSTSGGTAALGCLVEDYFPEPVTVSWNSGALTSGVHTFPAVLQSSGLYSLSSVVTVPSSSLGTQTYICNVNHKPSNTKVDEKVEPKSCDGGGGSGGGGSEVQLQESGPGLVKPSQSLSLTCSVTGYSITSGYYWNWIRQFPGNKLEWMGYITYDGSNNYNPSLKNRISITRDTSKNQFFLKLNSVTTEDTATYYCADFDYWGQGTTLTVSSASTKGPSVFPLAPSSKSTSGGTAALGCLVEDYFPEPVTVSWNSGALTSGVHTFPAVLQSSGLYSLSSVVTVPSSSLGTQTYICNVNHKPSNTKVDEKVEPKSCDGGGGSGGGGSDIQMTQSPSSLSASVGDRVTITCRASQDIRNYLNWYQQKPGKAPKLLIYYTSRLESGVPSRFSGSGSGTDYTLTISSLQPEDFATYYCQQGNTLPWTFGQGTKVEIKSSASTKGPSVFPLAPSSKSTSGGTAALGCLVKDYFPEPVTVSWNSGALTSGVHTFPAVLQSSGLYSLSSVVTVPSSSLGTQTYICNVNHKPSNTKVDKKVEPKSC

SEQ ID NO: 59 - protein, 229 aa, Artificial Sequence
  CD3 VH-CL
EVQLVESGGGLVQPGGSLRLSCAASGYSFTGYTMNWVRQAPGKGLEWVALINPYKGVSTYNQKFKDRFTISVDKSKNTAYLQMNSLRAEDTAVYYCARSGYYGDSDWYFDVWGQGTLVTVSSASVAAPSVFIFPPSDEQLKSGTASVVCLLNNFYPREAKVQWKVDNALQSGNSQESVTEQDSKDSTYSLSSTLTLSKADYEKHKVYACEVTHQGLSSPVTKSFNRGEC

SEQ ID NO: 60 - protein, 214 aa, Artificial Sequence
  MCSP VL-CL(RK)
DIVLTQSPSSLSASLGDRVTISCSASQGIRNYLNWYQQRPDGTVKLLIYYTSSLHSGVPSRFSGSGSGTDYSLTISNLEPEDIATYYCQQYSKLPWTFGGGTKLEIKRTVAAPSVFIFPPSDRKLKSGTASVVCLLNNFYPREAKVQWKVDNALQSGNSQESVTEQDSKDSTYSLSSTLTLSKADYEKHKVYACEVTHQGLSSPVTKSFNRGEC

SEQ ID NO: 61 - protein, 120 aa, Artificial Sequence [sequence omitted]

SEQ ID NO: 62 - protein, 107 aa, Artificial Sequence [sequence omitted]

SEQ ID NO: 63 - protein, 120 aa, Artificial Sequence
  Her3 VH
QVQLVQSGAEVKKPGASVKVSCKASGYTFRSSYISWVRQAPGQGLEWMGWIYAGTGSPSYNQKLQGRVTMTTDTSTSTAYMELRSLRSDDTAVYYCARHRDYYSNSLTYWGQGTLVTVSS

SEQ ID NO: 64 - protein, 113 aa, Artificial Sequence
  Her3 VL
DIVMTQSPDSLAVSLGERATINCKSSQSVLNSGNQKNYLTWYQQKPGQPPKLLIYWASTRESGVPDRFSGSGSGTDFTLTISSLQAEDVAVYYCQSDYSYPYTFGQGTKLEIK

SEQ ID NO: 65 - protein, 112 aa, Artificial Sequence
  MCSP VH
EVQLQESGPGLVKPSQSLSLTCSVTGYSITSGYYWNWIRQFPGNKLEWMGYITYDGSNNYNPSLKNRISITRDTSKNQFFLKLNSVTTEDTATYYCADFDYWGQGTTLTVSS

SEQ ID NO: 66 - protein, 107 aa, Artificial Sequence
  MCSP VL
DIVLTQSPSSLSASLGDRVTISCSASQGIRNYLNWYQQRPDGTVKLLIYYTSSLHSGVPSRFSGSGSGTDYSLTISNLEPEDIATYYCQQYSKLPWTFGGGTKLEIK

SEQ ID NO: 67 - protein, 19 aa, Artificial Sequence
  CD3 HCDR2
RIRSKYNNYATYYADSVKD

SEQ ID NO: 68 - protein, 14 aa, Artificial Sequence
  CD3 LCDR1
RSSTGAVTTSNYAN